European Patent Specification EP 4 060 029 B1, published January 1, 2025. Title: Novel protein variant and a method for producing L-lysine using the same. Applicant: CJ CheilJedang Corporation. The sequence listing filed with the application follows.

SEQUENCE LISTING (11 sequences)

SEQ ID NO: 1 - protein, 38 aa, Artificial Sequence
  (C33S)_NCgl3069_amino acid
MAVAKDVLSFSRPIPALHAIIGALGWFGMFAVSLWSTL

SEQ ID NO: 2 - DNA, 117 bp, Artificial Sequence
  (C33S)_NCgl3069_nucleic acid
gtggctgtcgcaaaagacgtgcttagtttttcacgacccattcccgcacttcacgccatcatcggcgcgcttggatggtttggaatgttcgcagttagtctgtggagcacgctgtaa

SEQ ID NO: 3 - protein, 38 aa, Artificial Sequence
  (WT)_NCgl3069_amino acid
MAVAKDVLSFSRPIPALHAIIGALGWFGMFAVCLWSTL

SEQ ID NO: 4 - DNA, 117 bp, Artificial Sequence
  (WT)_NCgl3069_nucleic acid
gtggctgtcgcaaaagacgtgcttagtttttcacgacccattcccgcacttcacgccatcatcggcgcgcttggatggtttggaatgttcgcagtttgtctgtggagcacgctgtaa

SEQ ID NO: 5 - DNA, 35 bp, Artificial Sequence
  NCgl3069_1F
tcgagctcggtaccctgccagccaatcacatggga

SEQ ID NO: 6 - DNA, 41 bp, Artificial Sequence
  NCgl3069_2R
ggtttggaatgttcgcagttagtctgtggagcacgctgtaa

SEQ ID NO: 7 - DNA, 41 bp, Artificial Sequence
  NCgl3069_3F
ttacagcgtgctccacagactaactgcgaacattccaaacc

SEQ ID NO: 8 - DNA, 35 bp, Artificial Sequence
  NCgl3069_4R
ctctagaggatccccaggccgggacactacgtgtg

SEQ ID NO: 9 - DNA, 20 bp, Artificial Sequence
  NCgl3069_5F
tgccagccaatcacatggga

SEQ ID NO: 10 - DNA, 20 bp, Artificial Sequence
  NCgl3069_6R
aggccgggacactacgtgtg

SEQ ID NO: 11 - DNA, 5803 bp, Artificial Sequence
  pDCM2_plasmid
gttcgcttgctgtccataaaaccgcccagtctagctatcgccatgtaagcccactgcaagctacctgctttctctttgcgcttgcgttttcccttgtccagatagcccagtagctgacattcatccggggtcagcaccgtttctgcggactggctttctacgtgttccgcttcctttagcagcccttgcgccctgagtgcttgcggcagcgtgaagctagcttttatcgccattcgccattcaggctgcgcaactgttgggaagggcgatcggtgcgggcctcttcgctattacgccagctggcgaaagggggatgtgctgcaaggcgattaagttgggtaacgccagggttttcccagtcacgacgttgtaaaacgacggccagtgaattcgagctcggtacccggggatcctctagagtcgacctgcaggcatgcaagcttggcgtaatcatggtcatagctgtttcctgtgtgaaattgttatccgctcacaattccacacaacatacgagccggaagcataaagtgtaaagcctggggtgcctaatgagtgagctaactcacattaattgcgttgcgctcactgcccgctttccagtcgggaaacctgtcgtgccagctgcattaatgaatcggccaacgcgcggggagaggcggtttgcgtattgggcgctcttccgcttcctcgctcactgactcgctgcgctcggtcgttcggctgcggcgagcggtatcagctcactcaaaggcggtaatacggttatccacagaatcaggggataacgcaggaaagaacatgtgagcaaaaggccagcaaaaggccaggaaccgtaaaaaggccgcgttgctggcgtttttccataggctccgcccccctgacgagcatcacaaaaatcgacgctcaagtcagaggtggcgaaacccgacaggactataaagataccaggcgtttccccctggaagctccctcgtgcgctctcctgttccgaccctgccgcttaccggatacctgtccgcctttctcccttcgggaagcgtggcgctttctcaatgctcacgctgtaggtatctcagttcggtgtaggtcgttcgctccaagctgggctgtgtgcacgaaccccccgttcagcccgaccgctgcgccttatccggtaactatcgtcttgagtccaacccggtaagacacgacttatcgccactggcagcagccactggtaacaggattagcagagcgaggtatgtaggcggtgctacagagttcttgaagtggtggcctaactacggctacactagaaggacagtatttggtatctgcgctctgctgaagccagttaccttcggaaaaagagttggtagctcttgatccggcaaacaaaccaccgctggtagcggtggtttttttgtttgcaagcagcagattacgcgcagaaaaaaaggatctcaagaagatcctttgatcttttctacggggtctgacgctcagtggaacgaaaactcacgttaagggattttggtcatgagattatcaaaaaggatcttcacctagatccttttggggtgggcgaagaactccagcatgagatccccgcgctggaggatcatccagccctgatagaaacagaagccactggagcacctcaaaaacaccatcatacactaaatcagtaagttggcagcatcacccgacgcactttgcgccgaataaatacctgtgacggaagatcacttcgcagaataaataaatcctggtgtccctgttgataccgggaagccctgggccaacttttggcgaaaatgagacgttgatcggcacgtaagaggttccaactttcaccataatgaaataagatcactaccgggcgtattttttgagttatcgagattttcaggagctgatagaaacagaagccactggagcacctcaaaaacaccatcatacactaaatcagtaagttggcagcatcacccgacgcactttgcgccgaataaatacctgtgacggaagatcacttcgcagaataaataaatcctggtgtccctgttgataccgggaagccctgggccaacttttggcgaaaatgagacgttgatcggcacgtaagaggttccaactttcaccataatgaaataagatcactaccgggcgtattttttgagttatcgagattttcaggagctctttggcatcgtctctcgcctgtcccctcagttcagtaatttcctgcatttgcctgtttccagtcggtagatattccacaaaacagcagggaagcagcgcttttccgctgcataaccctgcttcggggtcattatagcgattttttcggtatatccatcctttttcgcacgatatacaggattttgccaaagggttcgtgtagactttccttggtgtatccaacggcgtcagccgggcaggataggtgaagtaggcccacccgcgagcgggtgttccttcttcactgtcccttattcgcacctggcggtgctcaacgggaatcctgctctgcgaggctggccggctaccgccggcgtaacagatgagggcaagcggatggctgatgaaaccaagccaaccaggaagggcagcccacctatcaaggtgtactgccttccagacgaacgaagagcgattgaggaaaaggcggcggcggccggcatgagcctgtcggcctacctgctggccgtcggccagggctacaaaatcacgggcgtcgtggactatgagcacgtccgcgagggcgtcccggaaaacgattccgaagcccaacctttcatagaaggcggcggtggaatcgaaatctcgtgatggcaggttgggcgtcgcttggtcggtcatttcgaaaaaggttaggaatacggttagccatttgcctgcttttatatagttcantatgggattcacctttatgttgataagaaataaaagaaaatgccaataggatatcggcattttcttttgcgtttttatttgttaactgttaattgtccttgttcaaggatgctgtctttgacaacagatgttttcttgcctttgatgttcagcaggaagctcggcgcaaacgttgattgtttgtctgcgtagaatcctctgtttgtcatatagcttgtaatcacgacattgtttcctttcgcttgaggtacagcgaagtgtgagtaagtaaaggttacatcgttaggcggatcaagatccatttttaacacaaggccagttttgttcagcggcttgtatgggccagttaaagaattagaaacataaccaagcatgtaaatatcgttagacgtaatgccgtcaatcgtcatttttgatccgcgggagtcagtgaacaggtaccatttgccgttcattttaaagacgttcgcgcgttcaatttcatctgttactgtgttagatgcaatcagcggtttcatcacttttttcagtgtgtaatcatcgtttagctcaatcataccgagagcgccgtttgctaactcagccgtgcgttttttatcgctttgcagaagtttttgactttcttgacggaagaatgatgtgcttttgccatagtatgctttgttaaataaagattcttcgccttggtagccatcttcagttccagtgtttgcttcaaatactaagtatttgtggcctttatcttctacgtagtgaggatctctcagcgtatggttgtcgcctgagctgtagttgccttcatcgatgaactgctgtacattttgatacgtttttccgtcaccgtcaaagattgatttataatcctctacaccgttgatgttcaaagagctgtctgatgctgatacgttaacttgtgcagttgtcagtgtttgtttgccgtaatgtttaccggagaaatcagtgtagaataaacggatttttccgtcagatgtaaatgtggctgaacctgaccattcttgtgtttggtcttttaggatagaatcatttgcatcgaatttgtcgctgtctttaaagacgcggccagcgtttttccagctgtcaatagaagtttcgccgactttttgatagaacatgtaaatcgatgtgtcatccgcatttttaggatctccggctaatgcaaagacgatgtggtagccgtgatagtttgcgacagtgccgtcagcgttttgtaatggccagctgtcccaaacgtccaggccttttgcagaagagatatttttaattgtggacgaatcaaattcagaaacttgatatttttcatttttttgctgttcagggatttgcagcatatcatggcgtgtaatatgggaaatgccgtatgtttccttatatggcttttggttcgtttctttcgcaaacgcttgagttgcgcctcctgccagcagtgcggtagtaaaggttaatactgttgcttgttttgcaaactttttgatgttcatcgttcatgtctccttttttatgtactgtgttagcggtctgcttcttccagccctcctgtttgaagatggcaagttagttacgcacaataaaaaaagacctaaaatatgtaaggggtgacgccaaagtatacactttgccctttacacattttaggtcttgcctgctttatcagtaacaaacccgcgcgatttacttttcgacctcattctattagactctcgtttggattgcaactggtctattttcctcttttgtttgatagaaaatcataaaaggatttgcagactacgggcctaaagaactaaaaaatctatctgtttcttttcattctctgtattttttatagtttctgttgcatgggcataaagttgcctttttaatcacaattcagaaaatatcataatatctcatttcactaaataatagtgaacggcaggtatatgtgatgggttaaaaaggatcaccccagagtcccgctcagaagaactcgtcaagaaggcgatagaaggcgatgcgctgcgaatcgggagcggcgataccgtaaagcacgaggaagcggtcagcccattcgccgccaagctcttcagcaatatcacgggtagccaacgctatgtcctgatagcggtccgccacacccagccggccacagtcgatgaatccagaaaagcggccattttccaccatgatattcggcaagcaggcatcgccatgggtcacgacgagatcctcgccgtcgggcatccgcgccttgagcctggcgaacagttcggctggcgcgagcccctgatgctcttcgtccagatcatcctgatcgacaagaccggcttccatccgagtacgtgctcgctcgatgcgatgtttcgcttggtggtcgaatgggcaggtagccggatcaagcgtatgcagccgccgcattgcatcagccatgatggatactttctcggcaggagcaaggtgagatgacaggagatcctgccccggcacttcgcccaatagcagccagtcccttcccgcttcagtgacaacgtcgagacagctgcgcaaggaacgcccgtcgtggccagccacgatagccgcgctgcctcgtcttggagttcattcagggcaccggacaggtcggtcttgacaaaaagaaccgggcgcccctgcgctgacagccggaacacggcggcatcagagcagccgattgtctgttgtgcccagtcatagccgaatagcctctccacccaagcggccggagaacctgcgtgcaatccatcttgttcaatcatgcgaaacgatcctcatcctgtctcttgatcagatcttgatcccctgcgccatcagatccttggcggcaagaaagccatccagtttactttgcagggcttcccaaccttaccagagggcgccccagctggcaattccg